European Patent Application EP 4 477 674 A1, published December 18, 2024. Title: ENVIRONMENTALLY RESPONSIVE MASKED ANTIBODY AND USE THEREOF. Applicant: Daiichi Sankyo Company, Limited. Application EP 23752906.0, filed February 8, 2023. The sequence listing filed with the application follows.

SEQUENCE LISTING (81 sequences)

SEQ ID NO: 1 - protein, 470 aa, synthetic construct
  REGION 1..470: note = Amino acid sequence of the full length of HT1-11 H chain
MKHLWFFLLLVAAPRWVLSQVQLVQSGAEVKKPGASVKVSCKASGYTFTTAGMQWVRQAPGQGLEWMGWINTHSGVPKYAEDFKGRVTISADTSTSTAYLQLSSLKSEDTAVYYCARSGFGSSYWYFDVWGQGTLVTVSSASTKGPSVFPLAPSSKSTSGGTAALGCLVKDYFPEPVTVSWNSGALTSGVHTFPAVLQSSGLYSLSSVVTVPSSSLGTQTYICNVNHKPSNTKVDKRVEPKSCDKTHTCPPCPAPELLGGPSVFLFPPKPKDTLMISRTPEVTCVVVDVSHEDPEVKFNWYVDGVEVHNAKTKPREEQYNSTYRVVSVLTVLHQDWLNGKEYKCKVSNKALPAPIEKTISKAKGQPREPQVYTLPPSREEMTKNQVSLTCLVKGFYPSDIAVEWESNGQPENNYKTTPPVLDSDGSFFLYSKLTVDKSRWQQGNVFSCSVMHEALHNHYTQKSLSLSPGK

SEQ ID NO: 2 - protein, 234 aa, synthetic construct
  REGION 1..234: note = Amino acid sequence of the full length of HT1-11 L chain
MVLQTQVFISLLLWISGAYGDIQMTQSPSSLSASVGDRVTITCKASQDVSTAVAWYQQKPGKAPKLLIYSASYRYTGVPSRFSGSGSGTDFTLTISSLQPEDFAVYYCQQHYITPLTFGQGTKLEIKRTVAAPSVFIFPPSDEQLKSGTASVVCLLNNFYPREAKVQWKVDNALQSGNSQESVTEQDSKDSTYSLSSTLTLSKADYEKHKVYACEVTHQGLSSPVTKSFNRGEC

SEQ ID NO: 3 - protein, 331 aa, synthetic construct
  REGION 1..331: note = Amino acid sequence of the full length of MHT1001
MKYLLPTAAAGLLLLAAQPAMAAMGYLALKHPWPGLAENSGSGGGGSVLVPMAMMASGGSDVNSQVQLVQSGAEVKKPGASVKVSCKASGYTFTTAGMQWVRQAPGQGLEWMGWINTHSGVPKYAEDFKGRVTISADTSTSTAYLQLSSLKSEDTAVYYCARSGFGSSYWYFDVWGQGTLVTVSSGGGGSGGGGSGGGGSDIQMTQSPSSLSASVGDRVTITCKASQDVSTAVAWYQQKPGKAPKLLIYSASYRYTGVPSRFSGSGSGTDFTLTISSLQPEDFAVYYCQQHYITPLTFGQGTKLEIKRGAPSGDYKDDDDKGAAAHHHHHH

SEQ ID NO: 4 - protein, 331 aa, synthetic construct
  REGION 1..331: note = Amino acid sequence of the full length of MHT1002
MKYLLPTAAAGLLLLAAQPAMAAMGYLALKHPWPGLAENSGSGGGGSVLVPMAMMASGGSDVNSDIQMTQSPSSLSASVGDRVTITCKASQDVSTAVAWYQQKPGKAPKLLIYSASYRYTGVPSRFSGSGSGTDFTLTISSLQPEDFAVYYCQQHYITPLTFGQGTKLEIKRGGGGSGGGGSGGGGSQVQLVQSGAEVKKPGASVKVSCKASGYTFTTAGMQWVRQAPGQGLEWMGWINTHSGVPKYAEDFKGRVTISADTSTSTAYLQLSSLKSEDTAVYYCARSGFGSSYWYFDVWGQGTLVTVSSGAPSGDYKDDDDKGAAAHHHHHH

SEQ ID NO: 5 - protein, 294 aa, synthetic construct
  REGION 1..294: note = Amino acid sequence of the full length of HT1-11-scFv-HL
MKYLLPTAAAGLLLLAAQPAMAADVNSQVQLVQSGAEVKKPGASVKVSCKASGYTFTTAGMQWVRQAPGQGLEWMGWINTHSGVPKYAEDFKGRVTISADTSTSTAYLQLSSLKSEDTAVYYCARSGFGSSYWYFDVWGQGTLVTVSSGGGGSGGGGSGGGGSDIQMTQSPSSLSASVGDRVTITCKASQDVSTAVAWYQQKPGKAPKLLIYSASYRYTGVPSRFSGSGSGTDFTLTISSLQPEDFAVYYCQQHYITPLTFGQGTKLEIKRGAPSGDYKDDDDKGAAAHHHHHH

SEQ ID NO: 6 - protein, 294 aa, synthetic construct
  REGION 1..294: note = Amino acid sequence of the full length of HT1-11-scFv-LH
MKYLLPTAAAGLLLLAAQPAMAADVNSDIQMTQSPSSLSASVGDRVTITCKASQDVSTAVAWYQQKPGKAPKLLIYSASYRYTGVPSRFSGSGSGTDFTLTISSLQPEDFAVYYCQQHYITPLTFGQGTKLEIKRGGGGSGGGGSGGGGSQVQLVQSGAEVKKPGASVKVSCKASGYTFTTAGMQWVRQAPGQGLEWMGWINTHSGVPKYAEDFKGRVTISADTSTSTAYLQLSSLKSEDTAVYYCARSGFGSSYWYFDVWGQGTLVTVSSGAPSGDYKDDDDKGAAAHHHHHH

SEQ ID NO: 7 - protein, 506 aa, synthetic construct
  REGION 1..506: note = Amino acid sequence of the full length of MHT1007 H chain
MKHLWFFLLLVAAPRWVLSGYLALKHPWPGLAENSGSGGGGSVLVPMAMMASGGSQVQLVQSGAEVKKPGASVKVSCKASGYTFTTAGMQWVRQAPGQGLEWMGWINTHSGVPKYAEDFKGRVTISADTSTSTAYLQLSSLKSEDTAVYYCARSGFGSSYWYFDVWGQGTLVTVSSASTKGPSVFPLAPSSKSTSGGTAALGCLVKDYFPEPVTVSWNSGALTSGVHTFPAVLQSSGLYSLSSVVTVPSSSLGTQTYICNVNHKPSNTKVDKRVEPKSCDKTHTCPPCPAPELLGGPSVFLFPPKPKDTLMISRTPEVTCVVVDVSHEDPEVKFNWYVDGVEVHNAKTKPREEQYNSTYRVVSVLTVLHQDWLNGKEYKCKVSNKALPAPIEKTISKAKGQPREPQVYTLPPSREEMTKNQVSLTCLVKGFYPSDIAVEWESNGQPENNYKTTPPVLDSDGSFFLYSKLTVDKSRWQQGNVFSCSVMHEALHNHYTQKSLSLSPGK

SEQ ID NO: 8 - protein, 506 aa, synthetic construct
  REGION 1..506: note = Amino acid sequence of the full length of MHT1008 H chain
MKHLWFFLLLVAAPRWVLSGYLALKHPWPGLAENSGSGGGGSGGGGSGGGGSGGSQVQLVQSGAEVKKPGASVKVSCKASGYTFTTAGMQWVRQAPGQGLEWMGWINTHSGVPKYAEDFKGRVTISADTSTSTAYLQLSSLKSEDTAVYYCARSGFGSSYWYFDVWGQGTLVTVSSASTKGPSVFPLAPSSKSTSGGTAALGCLVKDYFPEPVTVSWNSGALTSGVHTFPAVLQSSGLYSLSSVVTVPSSSLGTQTYICNVNHKPSNTKVDKRVEPKSCDKTHTCPPCPAPELLGGPSVFLFPPKPKDTLMISRTPEVTCVVVDVSHEDPEVKFNWYVDGVEVHNAKTKPREEQYNSTYRVVSVLTVLHQDWLNGKEYKCKVSNKALPAPIEKTISKAKGQPREPQVYTLPPSREEMTKNQVSLTCLVKGFYPSDIAVEWESNGQPENNYKTTPPVLDSDGSFFLYSKLTVDKSRWQQGNVFSCSVMHEALHNHYTQKSLSLSPGK

SEQ ID NO: 9 - protein, 506 aa, synthetic construct
  REGION 1..506: note = Amino acid sequence of the full length of MHT1009 H chain
MKHLWFFLLLVAAPRWVLSGYLALKHPWPGLAENSGSGGSGGSGRSANAILEGGSQVQLVQSGAEVKKPGASVKVSCKASGYTFTTAGMQWVRQAPGQGLEWMGWINTHSGVPKYAEDFKGRVTISADTSTSTAYLQLSSLKSEDTAVYYCARSGFGSSYWYFDVWGQGTLVTVSSASTKGPSVFPLAPSSKSTSGGTAALGCLVKDYFPEPVTVSWNSGALTSGVHTFPAVLQSSGLYSLSSVVTVPSSSLGTQTYICNVNHKPSNTKVDKRVEPKSCDKTHTCPPCPAPELLGGPSVFLFPPKPKDTLMISRTPEVTCVVVDVSHEDPEVKFNWYVDGVEVHNAKTKPREEQYNSTYRVVSVLTVLHQDWLNGKEYKCKVSNKALPAPIEKTISKAKGQPREPQVYTLPPSREEMTKNQVSLTCLVKGFYPSDIAVEWESNGQPENNYKTTPPVLDSDGSFFLYSKLTVDKSRWQQGNVFSCSVMHEALHNHYTQKSLSLSPGK

SEQ ID NO: 10 - protein, 506 aa, synthetic construct
  REGION 1..506: note = Amino acid sequence of the full length of MHT1803 H chain
MKHLWFFLLLVAAPRWVLSGYLALKHPWPGLAEHHHSGGGGSGGGGSGGGGSHHHQVQLVQSGAEVKKPGASVKVSCKASGYTFTTAGMQWVRQAPGQGLEWMGWINTHSGVPKYAEDFKGRVTISADTSTSTAYLQLSSLKSEDTAVYYCARSGFGSSYWYFDVWGQGTLVTVSSASTKGPSVFPLAPSSKSTSGGTAALGCLVKDYFPEPVTVSWNSGALTSGVHTFPAVLQSSGLYSLSSVVTVPSSSLGTQTYICNVNHKPSNTKVDKRVEPKSCDKTHTCPPCPAPELLGGPSVFLFPPKPKDTLMISRTPEVTCVVVDVSHEDPEVKFNWYVDGVEVHNAKTKPREEQYNSTYRVVSVLTVLHQDWLNGKEYKCKVSNKALPAPIEKTISKAKGQPREPQVYTLPPSREEMTKNQVSLTCLVKGFYPSDIAVEWESNGQPENNYKTTPPVLDSDGSFFLYSKLTVDKSRWQQGNVFSCSVMHEALHNHYTQKSLSLSPGK

SEQ ID NO: 11 - protein, 506 aa, synthetic construct
  REGION 1..506: note = Amino acid sequence of the full length of MHT1804 H chain
MKHLWFFLLLVAAPRWVLSGYLALKHPWPGLAENSGSGHHHSGGGGSHHHGSGGSQVQLVQSGAEVKKPGASVKVSCKASGYTFTTAGMQWVRQAPGQGLEWMGWINTHSGVPKYAEDFKGRVTISADTSTSTAYLQLSSLKSEDTAVYYCARSGFGSSYWYFDVWGQGTLVTVSSASTKGPSVFPLAPSSKSTSGGTAALGCLVKDYFPEPVTVSWNSGALTSGVHTFPAVLQSSGLYSLSSVVTVPSSSLGTQTYICNVNHKPSNTKVDKRVEPKSCDKTHTCPPCPAPELLGGPSVFLFPPKPKDTLMISRTPEVTCVVVDVSHEDPEVKFNWYVDGVEVHNAKTKPREEQYNSTYRVVSVLTVLHQDWLNGKEYKCKVSNKALPAPIEKTISKAKGQPREPQVYTLPPSREEMTKNQVSLTCLVKGFYPSDIAVEWESNGQPENNYKTTPPVLDSDGSFFLYSKLTVDKSRWQQGNVFSCSVMHEALHNHYTQKSLSLSPGK

SEQ ID NO: 12 - protein, 506 aa, synthetic construct
  REGION 1..506: note = Amino acid sequence of the full length of MHT1805 H chain
MKHLWFFLLLVAAPRWVLSGYLALKHPWPGLAENSGSGGGGSHHHHSGGGGSGGSQVQLVQSGAEVKKPGASVKVSCKASGYTFTTAGMQWVRQAPGQGLEWMGWINTHSGVPKYAEDFKGRVTISADTSTSTAYLQLSSLKSEDTAVYYCARSGFGSSYWYFDVWGQGTLVTVSSASTKGPSVFPLAPSSKSTSGGTAALGCLVKDYFPEPVTVSWNSGALTSGVHTFPAVLQSSGLYSLSSVVTVPSSSLGTQTYICNVNHKPSNTKVDKRVEPKSCDKTHTCPPCPAPELLGGPSVFLFPPKPKDTLMISRTPEVTCVVVDVSHEDPEVKFNWYVDGVEVHNAKTKPREEQYNSTYRVVSVLTVLHQDWLNGKEYKCKVSNKALPAPIEKTISKAKGQPREPQVYTLPPSREEMTKNQVSLTCLVKGFYPSDIAVEWESNGQPENNYKTTPPVLDSDGSFFLYSKLTVDKSRWQQGNVFSCSVMHEALHNHYTQKSLSLSPGK

SEQ ID NO: 13 - protein, 506 aa, synthetic construct
  REGION 1..506: note = Amino acid sequence of the full length of MHT1806 H chain
MKHLWFFLLLVAAPRWVLSGYLALKHPWPGLAEHHHSGGGGSHHHHSGGGGSHHHQVQLVQSGAEVKKPGASVKVSCKASGYTFTTAGMQWVRQAPGQGLEWMGWINTHSGVPKYAEDFKGRVTISADTSTSTAYLQLSSLKSEDTAVYYCARSGFGSSYWYFDVWGQGTLVTVSSASTKGPSVFPLAPSSKSTSGGTAALGCLVKDYFPEPVTVSWNSGALTSGVHTFPAVLQSSGLYSLSSVVTVPSSSLGTQTYICNVNHKPSNTKVDKRVEPKSCDKTHTCPPCPAPELLGGPSVFLFPPKPKDTLMISRTPEVTCVVVDVSHEDPEVKFNWYVDGVEVHNAKTKPREEQYNSTYRVVSVLTVLHQDWLNGKEYKCKVSNKALPAPIEKTISKAKGQPREPQVYTLPPSREEMTKNQVSLTCLVKGFYPSDIAVEWESNGQPENNYKTTPPVLDSDGSFFLYSKLTVDKSRWQQGNVFSCSVMHEALHNHYTQKSLSLSPGK

SEQ ID NO: 14 - protein, 508 aa, synthetic construct
  REGION 1..508: note = Amino acid sequence of the full length of MHT1808 H chain
MKHLWFFLLLVAAPRWVLSGYLALKHPWPGLAENSGGGGSGHHHGGHHHGGHHHGGSQVQLVQSGAEVKKPGASVKVSCKASGYTFTTAGMQWVRQAPGQGLEWMGWINTHSGVPKYAEDFKGRVTISADTSTSTAYLQLSSLKSEDTAVYYCARSGFGSSYWYFDVWGQGTLVTVSSASTKGPSVFPLAPSSKSTSGGTAALGCLVKDYFPEPVTVSWNSGALTSGVHTFPAVLQSSGLYSLSSVVTVPSSSLGTQTYICNVNHKPSNTKVDKRVEPKSCDKTHTCPPCPAPELLGGPSVFLFPPKPKDTLMISRTPEVTCVVVDVSHEDPEVKFNWYVDGVEVHNAKTKPREEQYNSTYRVVSVLTVLHQDWLNGKEYKCKVSNKALPAPIEKTISKAKGQPREPQVYTLPPSREEMTKNQVSLTCLVKGFYPSDIAVEWESNGQPENNYKTTPPVLDSDGSFFLYSKLTVDKSRWQQGNVFSCSVMHEALHNHYTQKSLSLSPGK

SEQ ID NO: 15 - protein, 508 aa, synthetic construct
  REGION 1..508: note = Amino acid sequence of the full length of MHT1809 H chain
MKHLWFFLLLVAAPRWVLSGYLALKHPWPGLAENSGGGGSHHGGHHGGHHGGHHGGSQVQLVQSGAEVKKPGASVKVSCKASGYTFTTAGMQWVRQAPGQGLEWMGWINTHSGVPKYAEDFKGRVTISADTSTSTAYLQLSSLKSEDTAVYYCARSGFGSSYWYFDVWGQGTLVTVSSASTKGPSVFPLAPSSKSTSGGTAALGCLVKDYFPEPVTVSWNSGALTSGVHTFPAVLQSSGLYSLSSVVTVPSSSLGTQTYICNVNHKPSNTKVDKRVEPKSCDKTHTCPPCPAPELLGGPSVFLFPPKPKDTLMISRTPEVTCVVVDVSHEDPEVKFNWYVDGVEVHNAKTKPREEQYNSTYRVVSVLTVLHQDWLNGKEYKCKVSNKALPAPIEKTISKAKGQPREPQVYTLPPSREEMTKNQVSLTCLVKGFYPSDIAVEWESNGQPENNYKTTPPVLDSDGSFFLYSKLTVDKSRWQQGNVFSCSVMHEALHNHYTQKSLSLSPGK

SEQ ID NO: 16 - protein, 508 aa, synthetic construct
  REGION 1..508: note = Amino acid sequence of the full length of MHT1810 H chain
MKHLWFFLLLVAAPRWVLSGYLALKHPWPGLAENSGGGGHGHGHGHGHGHGHGHGGSQVQLVQSGAEVKKPGASVKVSCKASGYTFTTAGMQWVRQAPGQGLEWMGWINTHSGVPKYAEDFKGRVTISADTSTSTAYLQLSSLKSEDTAVYYCARSGFGSSYWYFDVWGQGTLVTVSSASTKGPSVFPLAPSSKSTSGGTAALGCLVKDYFPEPVTVSWNSGALTSGVHTFPAVLQSSGLYSLSSVVTVPSSSLGTQTYICNVNHKPSNTKVDKRVEPKSCDKTHTCPPCPAPELLGGPSVFLFPPKPKDTLMISRTPEVTCVVVDVSHEDPEVKFNWYVDGVEVHNAKTKPREEQYNSTYRVVSVLTVLHQDWLNGKEYKCKVSNKALPAPIEKTISKAKGQPREPQVYTLPPSREEMTKNQVSLTCLVKGFYPSDIAVEWESNGQPENNYKTTPPVLDSDGSFFLYSKLTVDKSRWQQGNVFSCSVMHEALHNHYTQKSLSLSPGK

SEQ ID NO: 17 - protein, 520 aa, synthetic construct
  REGION 1..520: note = Amino acid sequence of the full length of MHT1811 H chain
MKHLWFFLLLVAAPRWVLSGYLALKHPWPGLAENSGGGGSGGGSGHHHGGHHHGGHHHGSPLGLWAGGSQVQLVQSGAEVKKPGASVKVSCKASGYTFTTAGMQWVRQAPGQGLEWMGWINTHSGVPKYAEDFKGRVTISADTSTSTAYLQLSSLKSEDTAVYYCARSGFGSSYWYFDVWGQGTLVTVSSASTKGPSVFPLAPSSKSTSGGTAALGCLVKDYFPEPVTVSWNSGALTSGVHTFPAVLQSSGLYSLSSVVTVPSSSLGTQTYICNVNHKPSNTKVDKRVEPKSCDKTHTCPPCPAPELLGGPSVFLFPPKPKDTLMISRTPEVTCVVVDVSHEDPEVKFNWYVDGVEVHNAKTKPREEQYNSTYRVVSVLTVLHQDWLNGKEYKCKVSNKALPAPIEKTISKAKGQPREPQVYTLPPSREEMTKNQVSLTCLVKGFYPSDIAVEWESNGQPENNYKTTPPVLDSDGSFFLYSKLTVDKSRWQQGNVFSCSVMHEALHNHYTQKSLSLSPGK

SEQ ID NO: 18 - protein, 508 aa, synthetic construct
  REGION 1..508: note = Amino acid sequence of the full length of MHT1817 H chain
MKHLWFFLLLVAAPRWVLSGYLALKHPWPGLAENSGGGGSGHHHGGHDHGGHHHGGSQVQLVQSGAEVKKPGASVKVSCKASGYTFTTAGMQWVRQAPGQGLEWMGWINTHSGVPKYAEDFKGRVTISADTSTSTAYLQLSSLKSEDTAVYYCARSGFGSSYWYFDVWGQGTLVTVSSASTKGPSVFPLAPSSKSTSGGTAALGCLVKDYFPEPVTVSWNSGALTSGVHTFPAVLQSSGLYSLSSVVTVPSSSLGTQTYICNVNHKPSNTKVDKRVEPKSCDKTHTCPPCPAPELLGGPSVFLFPPKPKDTLMISRTPEVTCVVVDVSHEDPEVKFNWYVDGVEVHNAKTKPREEQYNSTYRVVSVLTVLHQDWLNGKEYKCKVSNKALPAPIEKTISKAKGQPREPQVYTLPPSREEMTKNQVSLTCLVKGFYPSDIAVEWESNGQPENNYKTTPPVLDSDGSFFLYSKLTVDKSRWQQGNVFSCSVMHEALHNHYTQKSLSLSPGK

SEQ ID NO: 19 - protein, 508 aa, synthetic construct
  REGION 1..508: note = Amino acid sequence of the full length of MHT1818 H chain
MKHLWFFLLLVAAPRWVLSGYLALKHPWPGLAENSGGGGSGHDHGGHHHGGHDHGGSQVQLVQSGAEVKKPGASVKVSCKASGYTFTTAGMQWVRQAPGQGLEWMGWINTHSGVPKYAEDFKGRVTISADTSTSTAYLQLSSLKSEDTAVYYCARSGFGSSYWYFDVWGQGTLVTVSSASTKGPSVFPLAPSSKSTSGGTAALGCLVKDYFPEPVTVSWNSGALTSGVHTFPAVLQSSGLYSLSSVVTVPSSSLGTQTYICNVNHKPSNTKVDKRVEPKSCDKTHTCPPCPAPELLGGPSVFLFPPKPKDTLMISRTPEVTCVVVDVSHEDPEVKFNWYVDGVEVHNAKTKPREEQYNSTYRVVSVLTVLHQDWLNGKEYKCKVSNKALPAPIEKTISKAKGQPREPQVYTLPPSREEMTKNQVSLTCLVKGFYPSDIAVEWESNGQPENNYKTTPPVLDSDGSFFLYSKLTVDKSRWQQGNVFSCSVMHEALHNHYTQKSLSLSPGK

SEQ ID NO: 20 - protein, 508 aa, synthetic construct
  REGION 1..508: note = Amino acid sequence of the full length of MHT1819 H chain
MKHLWFFLLLVAAPRWVLSGYLALKHPWPGLAENSGGGGSGHDHGGHDHGGHDHGGSQVQLVQSGAEVKKPGASVKVSCKASGYTFTTAGMQWVRQAPGQGLEWMGWINTHSGVPKYAEDFKGRVTISADTSTSTAYLQLSSLKSEDTAVYYCARSGFGSSYWYFDVWGQGTLVTVSSASTKGPSVFPLAPSSKSTSGGTAALGCLVKDYFPEPVTVSWNSGALTSGVHTFPAVLQSSGLYSLSSVVTVPSSSLGTQTYICNVNHKPSNTKVDKRVEPKSCDKTHTCPPCPAPELLGGPSVFLFPPKPKDTLMISRTPEVTCVVVDVSHEDPEVKFNWYVDGVEVHNAKTKPREEQYNSTYRVVSVLTVLHQDWLNGKEYKCKVSNKALPAPIEKTISKAKGQPREPQVYTLPPSREEMTKNQVSLTCLVKGFYPSDIAVEWESNGQPENNYKTTPPVLDSDGSFFLYSKLTVDKSRWQQGNVFSCSVMHEALHNHYTQKSLSLSPGK

SEQ ID NO: 21 - protein, 465 aa, synthetic construct
  REGION 1..465: note = Amino acid sequence of the full length of hM23H1L1 H chain
MKHLWFFLLLVAAPRWVLSQVQLVQSGAEVKKPGASVKVSCKASGYAFSNYLIEWVRQAPGQGLEWMGVINPGSGVTNYNEKFKGRVTITADTSTSTAYMELSSLRSEDTAVYYCARAEAWFAYWGQGTLVTVSSASTKGPSVFPLAPSSKSTSGGTAALGCLVKDYFPEPVTVSWNSGALTSGVHTFPAVLQSSGLYSLSSVVTVPSSSLGTQTYICNVNHKPSNTKVDKRVEPKSCDKTHTCPPCPAPELLGGPSVFLFPPKPKDTLMISRTPEVTCVVVDVSHEDPEVKFNWYVDGVEVHNAKTKPREEQYNSTYRVVSVLTVLHQDWLNGKEYKCKVSNKALPAPIEKTISKAKGQPREPQVYTLPPSREEMTKNQVSLTCLVKGFYPSDIAVEWESNGQPENNYKTTPPVLDSDGSFFLYSKLTVDKSRWQQGNVFSCSVMHEALHNHYTQKSLSLSPGK

SEQ ID NO: 22 - protein, 240 aa, synthetic construct
  REGION 1..240: note = Amino acid sequence of the full length of hM23H1L1 L chain
MVLQTQVFISLLLWISGAYGDIVMTQSPDSLAVSLGERATINCKSSQSLLYSSNQKNYLAWYQQKPGQPPKLLIYWASTRESGVPDRFSGSGSGTDFTLTISSLQAEDVAVYYCQRYYGYPWTFGQGTKVEIKRTVAAPSVFIFPPSDEQLKSGTASVVCLLNNFYPREAKVQWKVDNALQSGNSQESVTEQDSKDSTYSLSSTLTLSKADYEKHKVYACEVTHQGLSSPVTKSFNRGEC

SEQ ID NO: 23 - protein, 468 aa, synthetic construct
  REGION 1..468: note = Amino acid sequence of the full length of Cetuximab H chain
MKHLWFFLLLVAAPRWVLSQVQLKQSGPGLVQPSQSLSITCTVSGFSLTNYGVHWVRQSPGKGLEWLGVIWSGGNTDYNTPFTSRLSINKDNSKSQVFFKMNSLQSNDTAIYYCARALTYYDYEFAYWGQGTLVTVSAASTKGPSVFPLAPSSKSTSGGTAALGCLVKDYFPEPVTVSWNSGALTSGVHTFPAVLQSSGLYSLSSVVTVPSSSLGTQTYICNVNHKPSNTKVDKRVEPKSCDKTHTCPPCPAPELLGGPSVFLFPPKPKDTLMISRTPEVTCVVVDVSHEDPEVKFNWYVDGVEVHNAKTKPREEQYNSTYRVVSVLTVLHQDWLNGKEYKCKVSNKALPAPIEKTISKAKGQPREPQVYTLPPSREEMTKNQVSLTCLVKGFYPSDIAVEWESNGQPENNYKTTPPVLDSDGSFFLYSKLTVDKSRWQQGNVFSCSVMHEALHNHYTQKSLSLSPGK

SEQ ID NO: 24 - protein, 234 aa, synthetic construct
  REGION 1..234: note = Amino acid sequence of the full length of Cetuximab L chain
MVLQTQVFISLLLWISGAYGDILLTQSPVILSVSPGERVSFSCRASQSIGTNIHWYQQRTNGSPRLLIKYASESISGIPSRFSGSGSGTDFTLSINSVESEDIADYYCQQNNNWPTTFGAGTKLELKRTVAAPSVFIFPPSDEQLKSGTASVVCLLNNFYPREAKVQWKVDNALQSGNSQESVTEQDSKDSTYSLSSTLTLSKADYEKHKVYACEVTHQGLSSPVTKSFNRGEC

SEQ ID NO: 25 - protein, 464 aa, synthetic construct
  REGION 1..464: note = Amino acid sequence of the full length of C3022 H chain
MKHLWFFLLLVAAPRWVLSQVQLVQSGAEVKKPGASVKVSCKASGYTFTGYYMHWVRQAPGQGLEWMGRINPNSGGTNYAQKFQGRVTMTRDTSISTAYMELSGLRSDDTAVYYCASGSVRHPWGQGTLVTVSSASTKGPSVFPLAPSSKSTSGGTAALGCLVKDYFPEPVTVSWNSGALTSGVHTFPAVLQSSGLYSLSSVVTVPSSSLGTQTYICNVNHKPSNTKVDKRVEPKSCDKTHTCPPCPAPELLGGPSVFLFPPKPKDTLMISRTPEVTCVVVDVSHEDPEVKFNWYVDGVEVHNAKTKPREEQYNSTYRVVSVLTVLHQDWLNGKEYKCKVSNKALPAPIEKTISKAKGQPREPQVYTLPPSREEMTKNQVSLTCLVKGFYPSDIAVEWESNGQPENNYKTTPPVLDSDGSFFLYSKLTVDKSRWQQGNVFSCSVMHEALHNHYTQKSLSLSPGK

SEQ ID NO: 26 - protein, 236 aa, synthetic construct
  REGION 1..236: note = Amino acid sequence of the full length of C3022 L chain
MVLQTQVFISLLLWISGAYGQPVLTQPPSASGTPGQRVTISCSGSRSNIGGNIVSWYQQFPGTAPRLLTYADNQRPSGVPDRFSGSKSGTSASLAISGLQSEDEADYYCAAWDDSLNGVVFGGGTKLTVLGQPKAAPSVTLFPPSSEELQANKATLVCLISDFYPGAVTVAWKADSSPVKAGVETTTPSKQSNNKYAASSYLSLTPEQWKSHRSYSCQVTHEGSTVEKTVAPTECS

SEQ ID NO: 27 - protein, 278 aa, synthetic construct
  REGION 1..278: note = Amino acid sequence of the full length of MhM8001 L chain
MVLQTQVFISLLLWISGAYGGENMWNDLDLVPLGILGGGGSGHHHGGHHHGGHHHGGSDIVMTQSPDSLAVSLGERATINCKSSQSLLYSSNQKNYLAWYQQKPGQPPKLLIYWASTRESGVPDRFSGSGSGTDFTLTISSLQAEDVAVYYCQRYYGYPWTFGQGTKVEIKRTVAAPSVFIFPPSDEQLKSGTASVVCLLNNFYPREAKVQWKVDNALQSGNSQESVTEQDSKDSTYSLSSTLTLSKADYEKHKVYACEVTHQGLSSPVTKSFNRGEC

SEQ ID NO: 28 - protein, 273 aa, synthetic construct
  REGION 1..273: note = Amino acid sequence of the full length of MCE-2101 L chain
MVLQTQVFISLLLWISGAYGMGLMHMEKSRSWYLSRQGGGGSGHHHGGHHHGGHHHGGSDILLTQSPVILSVSPGERVSFSCRASQSIGTNIHWYQQRTNGSPRLLIKYASESISGIPSRFSGSGSGTDFTLSINSVESEDIADYYCQQNNNWPTTFGAGTKLELKRTVAAPSVFIFPPSDEQLKSGTASVVCLLNNFYPREAKVQWKVDNALQSGNSQESVTEQDSKDSTYSLSSTLTLSKADYEKHKVYACEVTHQGLSSPVTKSFNRGEC

SEQ ID NO: 29 - protein, 502 aa, synthetic construct
  REGION 1..502: note = Amino acid sequence of the full length of MC3-9001 H chain
MKHLWFFLLLVAAPRWVLSGETMSVFTRDYFTETPGGGGSGHHHGGHHHGGHHHGGSQVQLVQSGAEVKKPGASVKVSCKASGYTFTGYYMHWVRQAPGQGLEWMGRINPNSGGTNYAQKFQGRVTMTRDTSISTAYMELSGLRSDDTAVYYCASGSVRHPWGQGTLVTVSSASTKGPSVFPLAPSSKSTSGGTAALGCLVKDYFPEPVTVSWNSGALTSGVHTFPAVLQSSGLYSLSSVVTVPSSSLGTQTYICNVNHKPSNTKVDKRVEPKSCDKTHTCPPCPAPELLGGPSVFLFPPKPKDTLMISRTPEVTCVVVDVSHEDPEVKFNWYVDGVEVHNAKTKPREEQYNSTYRVVSVLTVLHQDWLNGKEYKCKVSNKALPAPIEKTISKAKGQPREPQVYTLPPSREEMTKNQVSLTCLVKGFYPSDIAVEWESNGQPENNYKTTPPVLDSDGSFFLYSKLTVDKSRWQQGNVFSCSVMHEALHNHYTQKSLSLSPGK

SEQ ID NO: 30 - protein, 506 aa, synthetic construct
  REGION 1..506: note = Amino acid sequence of the full length of MHT1221 H chain
MKHLWFFLLLVAAPRWVLSGYLALKHPWPGLASGSGSGGGGSGGGGSGGGGSGGSQVQLVQSGAEVKKPGASVKVSCKASGYTFTTAGMQWVRQAPGQGLEWMGWINTHSGVPKYAEDFKGRVTISADTSTSTAYLQLSSLKSEDTAVYYCARSGFGSSYWYFDVWGQGTLVTVSSASTKGPSVFPLAPSSKSTSGGTAALGCLVKDYFPEPVTVSWNSGALTSGVHTFPAVLQSSGLYSLSSVVTVPSSSLGTQTYICNVNHKPSNTKVDKRVEPKSCDKTHTCPPCPAPELLGGPSVFLFPPKPKDTLMISRTPEVTCVVVDVSHEDPEVKFNWYVDGVEVHNAKTKPREEQYNSTYRVVSVLTVLHQDWLNGKEYKCKVSNKALPAPIEKTISKAKGQPREPQVYTLPPSREEMTKNQVSLTCLVKGFYPSDIAVEWESNGQPENNYKTTPPVLDSDGSFFLYSKLTVDKSRWQQGNVFSCSVMHEALHNHYTQKSLSLSPGK

SEQ ID NO: 31 - protein, 465 aa, synthetic construct
  REGION 1..465: note = Amino acid sequence of the full length of hM23-M1 H chain
MKHLWFFLLLVAAPRWVLSQVQLVQSGAEVKKPGASVKVSCKASGAAFSNYLIEWVRQAPGQGLEWMGVINPGSGVTNYNEKFKGRVTITADTSTSTAYMELSSLRSEDTAVYYCARAEAWFAYWGQGTLVTVSSASTKGPSVFPLAPSSKSTSGGTAALGCLVKDYFPEPVTVSWNSGALTSGVHTFPAVLQSSGLYSLSSVVTVPSSSLGTQTYICNVNHKPSNTKVDKRVEPKSCDKTHTCPPCPAPELLGGPSVFLFPPKPKDTLMISRTPEVTCVVVDVSHEDPEVKFNWYVDGVEVHNAKTKPREEQYNSTYRVVSVLTVLHQDWLNGKEYKCKVSNKALPAPIEKTISKAKGQPREPQVYTLPPSREEMTKNQVSLTCLVKGFYPSDIAVEWESNGQPENNYKTTPPVLDSDGSFFLYSKLTVDKSRWQQGNVFSCSVMHEALHNHYTQKSLSLSPGK

SEQ ID NO: 32 - protein, 240 aa, synthetic construct
  REGION 1..240: note = Amino acid sequence of the full length of hM23-M1 L chain
MVLQTQVFISLLLWISGAYGDIVMTQSPDSLAVSLGERATINCKSSQSLLYSSNQKNYLAWYQQKPGQPPKLLIYWASTRESGVPDRFSGSGSGTDFTLTISSLQAEDVAVYYCQRYYGYPWTFGQGTKVEIKRAVAAPSVFIFPPSDEQLKSGTASVVCLLNNFYPREAKVQWKVDNALQSGNSQESVTEQDSKDSTYSLSSTLTLSKADYEKHKVYACEVTHQGLSSPVTKSFNRGEC

SEQ ID NO: 33 - protein, 276 aa, synthetic construct
  REGION 1..276: note = Amino acid sequence of the full length of MhM1013 L chain
MVLQTQVFISLLLWISGAYGGNFYHQYPWPLEILGSGSGGGGSVLVPMAMMASGGSDIVMTQSPDSLAVSLGERATINCKSSQSLLYSSNQKNYLAWYQQKPGQPPKLLIYWASTRESGVPDRFSGSGSGTDFTLTISSLQAEDVAVYYCQRYYGYPWTFGQGTKVEIKRTVAAPSVFIFPPSDEQLKSGTASVVCLLNNFYPREAKVQWKVDNALQSGNSQESVTEQDSKDSTYSLSSTLTLSKADYEKHKVYACEVTHQGLSSPVTKSFNRGEC

SEQ ID NO: 34 - protein, 276 aa, synthetic construct
  REGION 1..276: note = Amino acid sequence of the full length of MhM1018-M1 L chain
MVLQTQVFISLLLWISGAYGGNFYHQYPWPLEILGSGSGGGGSGGGGSGGGGSGGSDIVMTQSPDSLAVSLGERATINCKSSQSLLYSSNQKNYLAWYQQKPGQPPKLLIYWASTRESGVPDRFSGSGSGTDFTLTISSLQAEDVAVYYCQRYYGYPWTFGQGTKVEIKRTVAAPSVFIFPPSDEQLKSGTASVVCLLNNFYPREAKVQWKVDNALQSGNSQESVTEQDSKDSTYSLSSTLTLSKADYEKHKVYACEVTHQGLSSPVTKSFNRGEC

SEQ ID NO: 35 - protein, 278 aa, synthetic construct
  REGION 1..278: note = Amino acid sequence of the full length of MhM1024-M1 L chain
MVLQTQVFISLLLWISGAYGGNFYHQYPWPLEILGSGGGGSGHHHGGHHHGGHHHGGSDIVMTQSPDSLAVSLGERATINCKSSQSLLYSSNQKNYLAWYQQKPGQPPKLLIYWASTRESGVPDRFSGSGSGTDFTLTISSLQAEDVAVYYCQRYYGYPWTFGQGTKVEIKRTVAAPSVFIFPPSDEQLKSGTASVVCLLNNFYPREAKVQWKVDNALQSGNSQESVTEQDSKDSTYSLSSTLTLSKADYEKHKVYACEVTHQGLSSPVTKSFNRGEC

SEQ ID NO: 36 - protein, 10 aa, synthetic construct
  REGION 1..10: note = Synthetic
SGRSANAILE

SEQ ID NO: 37 - protein, 7 aa, synthetic construct
  REGION 1..7: note = Synthetic
SGRSANA

SEQ ID NO: 38 - protein, 5 aa, synthetic construct
  REGION 1..5: note = Synthetic
SGRSA

SEQ ID NO: 39 - protein, 10 aa, synthetic construct
  REGION 1..10: note = Synthetic
VLVPMAMMAS

SEQ ID NO: 40 - protein, 6 aa, synthetic construct
  REGION 1..6: note = Synthetic
PLGLWA

SEQ ID NO: 41 - protein, 6 aa, synthetic construct
  REGION 1..6: note = Synthetic
PLGLAG

SEQ ID NO: 42 - protein, 22 aa, synthetic construct
  REGION 1..22: note = Synthetic
GGGGSHHGGHHGGHHGGHHGGS

SEQ ID NO: 43 - protein, 24 aa, synthetic construct
  REGION 1..24: note = Synthetic
GGGGSHHGGHRHGGHHKGGHHGGS

SEQ ID NO: 44 - protein, 23 aa, synthetic construct
  REGION 1..23: note = Synthetic
GGGGSHGHGHGHGHGHGHGHGGS

SEQ ID NO: 45 - protein, 27 aa, synthetic construct
  REGION 1..27: note = Synthetic
MYKDCIESTGDYFLLCDAEGPWGIILE

SEQ ID NO: 46 - protein, 20 aa, synthetic construct
  REGION 1..20: note = Synthetic
GSGGGGSVLVPMAMMASGGS

SEQ ID NO: 47 - protein, 20 aa, synthetic construct
  REGION 1..20: note = Synthetic
GSGGGGSGGGGSGGGGSGGS

SEQ ID NO: 48 - protein, 20 aa, synthetic construct
  REGION 1..20: note = Synthetic
GSGGSGGSGRSANAILEGGS

SEQ ID NO: 49 - protein, 22 aa, synthetic construct
  REGION 1..22: note = Synthetic
HHHSGGGGSGGGGSGGGGSHHH

SEQ ID NO: 50 - protein, 20 aa, synthetic construct
  REGION 1..20: note = Synthetic
GSGHHHSGGGGSHHHGSGGS

SEQ ID NO: 51 - protein, 20 aa, synthetic construct
  REGION 1..20: note = Synthetic
GSGGGGSHHHHSGGGGSGGS

SEQ ID NO: 52 - protein, 22 aa, synthetic construct
  REGION 1..22: note = Synthetic
HHHSGGGGSHHHHSGGGGSHHH

SEQ ID NO: 53 - protein, 22 aa, synthetic construct
  REGION 1..22: note = Synthetic
GGGGSGHHHGGHHHGGHHHGGS

SEQ ID NO: 54 - protein, 22 aa, synthetic construct
  REGION 1..22: note = Synthetic
GGGGHGHGHGHGHGHGHGHGGS

SEQ ID NO: 55 - protein, 34 aa, synthetic construct
  REGION 1..34: note = Synthetic
GGGGSGGGSGHHHGGHHHGGHHHGSPLGLWAGGS

SEQ ID NO: 56 - protein, 22 aa, synthetic construct
  REGION 1..22: note = Synthetic
GGGGSGHHHGGHDHGGHHHGGS

SEQ ID NO: 57 - protein, 22 aa, synthetic construct
  REGION 1..22: note = Synthetic
GGGGSGHDHGGHHHGGHDHGGS

SEQ ID NO: 58 - protein, 22 aa, synthetic construct
  REGION 1..22: note = Synthetic
GGGGSGHDHGGHDHGGHDHGGS

SEQ ID NO: 59 - protein, 22 aa, synthetic construct
  REGION 1..22: note = Synthetic
GGGGSGHHHGGHHHGGHHHGGS

SEQ ID NO: 60 - protein, 22 aa, synthetic construct
  REGION 1..22: note = Synthetic
GGGGSGHHHGGHHHGGHHHGGS

SEQ ID NO: 61 - protein, 22 aa, synthetic construct
  REGION 1..22: note = Synthetic
GGGGSGHHHGGHHHGGHHHGGS

SEQ ID NO: 62 - protein, 20 aa, synthetic construct
  REGION 1..20: note = Synthetic
GSGGGGSGGGGSGGGGSGGS

SEQ ID NO: 63 - protein, 22 aa, synthetic construct
  REGION 1..22: note = Synthetic
GSGSGGGGSVLVPMAMMASGGS

SEQ ID NO: 64 - protein, 22 aa, synthetic construct
  REGION 1..22: note = Synthetic
GSGSGGGGSGGGGSGGGGSGGS

SEQ ID NO: 65 - protein, 24 aa, synthetic construct
  REGION 1..24: note = Synthetic
GSGGGGSGHHHGGHHHGGHHHGGS

SEQ ID NO: 66 - protein, 22 aa, synthetic construct
  REGION 1..22: note = Synthetic
GGGGSGHHHGGHRHGGHHHGGS

SEQ ID NO: 67 - protein, 6 aa, synthetic construct
  REGION 1..6: note = Synthetic
PLFAAP

SEQ ID NO: 68 - protein, 280 aa, synthetic construct
  REGION 1..280: note = Amino acid sequence of the full length of MhM1026-M1 L chain
MVLQTQVFISLLLWISGAYGGNFYHQYPWPLEILGSGGGGSGGGHHHGGHHHGGHHHGGSDIVMTQSPDSLAVSLGERATINCKSSQSLLYSSNQKNYLAWYQQKPGQPPKLLIYWASTRESGVPDRFSGSGSGTDFTLTISSLQAEDVAVYYCQRYYGYPWTFGQGTKVEIKRTVAAPSVFIFPPSDEQLKSGTASVVCLLNNFYPREAKVQWKVDNALQSGNSQESVTEQDSKDSTYSLSSTLTLSKADYEKHKVYACEVTHQGLSSPVTKSFNRGEC

SEQ ID NO: 69 - protein, 280 aa, synthetic construct
  REGION 1..280: note = Amino acid sequence of the full length of MhM1028-M1 L chain
MVLQTQVFISLLLWISGAYGGNFYHQYPWPLEILGSGGGGSGGGHHHGRHHHGGHHHGGSDIVMTQSPDSLAVSLGERATINCKSSQSLLYSSNQKNYLAWYQQKPGQPPKLLIYWASTRESGVPDRFSGSGSGTDFTLTISSLQAEDVAVYYCQRYYGYPWTFGQGTKVEIKRTVAAPSVFIFPPSDEQLKSGTASVVCLLNNFYPREAKVQWKVDNALQSGNSQESVTEQDSKDSTYSLSSTLTLSKADYEKHKVYACEVTHQGLSSPVTKSFNRGEC

SEQ ID NO: 70 - protein, 280 aa, synthetic construct
  REGION 1..280: note = Amino acid sequence of the full length of MhM1042-M1 L chain
MVLQTQVFISLLLWISGAYGGNFYHQYPWPLEILGSGGGGSGGRHHHGGHHHGGHHHGGSDIVMTQSPDSLAVSLGERATINCKSSQSLLYSSNQKNYLAWYQQKPGQPPKLLIYWASTRESGVPDRFSGSGSGTDFTLTISSLQAEDVAVYYCQRYYGYPWTFGQGTKVEIKRTVAAPSVFIFPPSDEQLKSGTASVVCLLNNFYPREAKVQWKVDNALQSGNSQESVTEQDSKDSTYSLSSTLTLSKADYEKHKVYACEVTHQGLSSPVTKSFNRGEC

SEQ ID NO: 71 - protein, 280 aa, synthetic construct
  REGION 1..280: note = Amino acid sequence of the full length of MhM1043-M1 L chain
MVLQTQVFISLLLWISGAYGGNFYHQYPWPLEILGSGGGGSGGGHHHGGHHHGRHHHGGSDIVMTQSPDSLAVSLGERATINCKSSQSLLYSSNQKNYLAWYQQKPGQPPKLLIYWASTRESGVPDRFSGSGSGTDFTLTISSLQAEDVAVYYCQRYYGYPWTFGQGTKVEIKRTVAAPSVFIFPPSDEQLKSGTASVVCLLNNFYPREAKVQWKVDNALQSGNSQESVTEQDSKDSTYSLSSTLTLSKADYEKHKVYACEVTHQGLSSPVTKSFNRGEC

SEQ ID NO: 72 - protein, 280 aa, synthetic construct
  REGION 1..280: note = Amino acid sequence of the full length of MhM1044-M1 L chain
MVLQTQVFISLLLWISGAYGGNFYHQYPWPLEILGSGGGGSGGGHHHGKHHHGGHHHGGSDIVMTQSPDSLAVSLGERATINCKSSQSLLYSSNQKNYLAWYQQKPGQPPKLLIYWASTRESGVPDRFSGSGSGTDFTLTISSLQAEDVAVYYCQRYYGYPWTFGQGTKVEIKRTVAAPSVFIFPPSDEQLKSGTASVVCLLNNFYPREAKVQWKVDNALQSGNSQESVTEQDSKDSTYSLSSTLTLSKADYEKHKVYACEVTHQGLSSPVTKSFNRGEC

SEQ ID NO: 73 - protein, 280 aa, synthetic construct
  REGION 1..280: note = Amino acid sequence of the full length of MhM1045-M1 L chain
MVLQTQVFISLLLWISGAYGGNFYHQYPWPLEILGSGGGGSGGKHHHGGHHHGGHHHGGSDIVMTQSPDSLAVSLGERATINCKSSQSLLYSSNQKNYLAWYQQKPGQPPKLLIYWASTRESGVPDRFSGSGSGTDFTLTISSLQAEDVAVYYCQRYYGYPWTFGQGTKVEIKRTVAAPSVFIFPPSDEQLKSGTASVVCLLNNFYPREAKVQWKVDNALQSGNSQESVTEQDSKDSTYSLSSTLTLSKADYEKHKVYACEVTHQGLSSPVTKSFNRGEC

SEQ ID NO: 74 - protein, 280 aa, synthetic construct
  REGION 1..280: note = Amino acid sequence of the full length of MhM1046-M1 L chain
MVLQTQVFISLLLWISGAYGGNFYHQYPWPLEILGSGGGGSGGGHHHGGHHHGKHHHGGSDIVMTQSPDSLAVSLGERATINCKSSQSLLYSSNQKNYLAWYQQKPGQPPKLLIYWASTRESGVPDRFSGSGSGTDFTLTISSLQAEDVAVYYCQRYYGYPWTFGQGTKVEIKRTVAAPSVFIFPPSDEQLKSGTASVVCLLNNFYPREAKVQWKVDNALQSGNSQESVTEQDSKDSTYSLSSTLTLSKADYEKHKVYACEVTHQGLSSPVTKSFNRGEC

SEQ ID NO: 75 - protein, 24 aa, synthetic construct
  REGION 1..24: note = Synthetic
GGGGSGGGHHHGGHHHGGHHHGGS

SEQ ID NO: 76 - protein, 24 aa, synthetic construct
  REGION 1..24: note = Synthetic
GGGGSGGGHHHGRHHHGGHHHGGS

SEQ ID NO: 77 - protein, 24 aa, synthetic construct
  REGION 1..24: note = Synthetic
GGGGSGGRHHHGGHHHGGHHHGGS

SEQ ID NO: 78 - protein, 24 aa, synthetic construct
  REGION 1..24: note = Synthetic
GGGGSGGGHHHGGHHHGRHHHGGS

SEQ ID NO: 79 - protein, 24 aa, synthetic construct
  REGION 1..24: note = Synthetic
GGGGSGGGHHHGKHHHGGHHHGGS

SEQ ID NO: 80 - protein, 24 aa, synthetic construct
  REGION 1..24: note = Synthetic
GGGGSGGKHHHGGHHHGGHHHGGS

SEQ ID NO: 81 - protein, 24 aa, synthetic construct
  REGION 1..24: note = Synthetic
GGGGSGGGHHHGGHHHGKHHHGGS